European Patent Application EP 4 585 606 A1, published July 16, 2025. Title: OLIGOPEPTIDE AND USE AND COMPOSITION THEREOF. Applicant: Buddhist Tzu Chi Medical Foundation, Hualien, TAIWAN. Application US. The sequence listing filed with the application follows.

SEQUENCE LISTING (16 sequences)

SEQ ID NO: 1 - protein, 5 aa, synthetic construct
TSKYR

SEQ ID NO: 2 - protein, 4 aa, synthetic construct
TSKY

SEQ ID NO: 3 - DNA, 20 bp, synthetic construct
  source 1..20: mol_type = other DNA
cacctccccaacagatgctt

SEQ ID NO: 4 - DNA, 20 bp, synthetic construct
  source 1..20: mol_type = other DNA
ggtacttgttccagccctcc

SEQ ID NO: 5 - DNA, 22 bp, synthetic construct
  source 1..22: mol_type = other DNA
tgctgcccagatggctggagga

SEQ ID NO: 6 - DNA, 22 bp, synthetic construct
  source 1..22: mol_type = other DNA
tgccttgaaatccttgaggccc

SEQ ID NO: 7 - DNA, 20 bp, synthetic construct
  source 1..20: mol_type = other DNA
agagctacgagctgcctgac

SEQ ID NO: 8 - DNA, 19 bp, synthetic construct
  source 1..19: mol_type = other DNA
agcactgtgttggcgtaca

SEQ ID NO: 9 - DNA, 21 bp, synthetic construct
  source 1..21: mol_type = other DNA
tacttcgtcagcatcctatca

SEQ ID NO: 10 - DNA, 18 bp, synthetic construct
  source 1..18: mol_type = other DNA
ttccgtcagcgtcaacac

SEQ ID NO: 11 - DNA, 20 bp, synthetic construct
  source 1..20: mol_type = other DNA
gagggcaataaggtagtgaa

SEQ ID NO: 12 - DNA, 19 bp, synthetic construct
  source 1..19: mol_type = other DNA
catagatgcgtttgtaggc

SEQ ID NO: 13 - DNA, 21 bp, synthetic construct
  source 1..21: mol_type = other DNA
gagaaggagatcacggcttcc

SEQ ID NO: 14 - DNA, 20 bp, synthetic construct
  source 1..20: mol_type = other DNA
aagtctggcttcttggtcgt

SEQ ID NO: 15 - DNA, 18 bp, synthetic construct
  source 1..18: mol_type = other DNA
gcctcctcggagtccttg

SEQ ID NO: 16 - DNA, 19 bp, synthetic construct
  source 1..19: mol_type = other DNA
cgaagaccaactgctcgtg